European Patent Application EP 4 768 598 A1, published July 1, 2026. Title: 複数のライブラリを用いたペプチドのスクリーニング方法. Applicant: 中外製薬株式会社. The sequence listing filed with the application follows.

SEQUENCE LISTING (30 sequences)

SEQ ID NO: 1 - DNA, 104 bp, synthetic construct
  source 1..104: mol_type = other DNA
gtaatacgactcactatagggttaactttaataaggagatataaatatgnnnnnnnnnnnnnnnnnnnnnnnntagccgaccggcaccggcaccggcaaaaaaa

SEQ ID NO: 2 - DNA, 107 bp, synthetic construct
  source 1..107: mol_type = other DNA
gtaatacgactcactatagggttaactttaataaggagatataaatatgnnnnnnnnnnnnnnnnnnnnnnnnnnntagccgaccggcaccggcaccggcaaaaaaa

SEQ ID NO: 3 - DNA, 28 bp, synthetic construct
  source 1..28: mol_type = other DNA
tttttttgccggtgccggtgccggtcgg

SEQ ID NO: 4 - DNA, 60 bp, synthetic construct
  source 1..60: mol_type = other DNA
aaacacgtggcaaacattccaagaattactgacccctcggtttttttgccggtgccggtg

SEQ ID NO: 5 - DNA, 60 bp, synthetic construct
  source 1..60: mol_type = other DNA
aaacacgtggcaaacattccaaagcactcttaggcctctgtttttttgccggtgccggtg

SEQ ID NO: 6 - DNA, 60 bp, synthetic construct
  source 1..60: mol_type = other DNA
aaacacgtggcaaacattccaaggactgcataccaggttgtttttttgccggtgccggtg

SEQ ID NO: 7 - DNA, 60 bp, synthetic construct
  source 1..60: mol_type = other DNA
aaacacgtggcaaacattccaaggcccagaaggatacaactttttttgccggtgccggtg

SEQ ID NO: 8 - DNA, 38 bp, synthetic construct
  source 1..38: mol_type = other DNA
gtaatacgactcactatagggttaactttaataaggag

SEQ ID NO: 9 - DNA, 31 bp, synthetic construct
  source 1..31: mol_type = other DNA
tttttttgccggtgccggtgccggtcggcta

SEQ ID NO: 10 - DNA, 29 bp, synthetic construct
  source 1..29: mol_type = other DNA
tttgtggtgccggtgccggtgccggtcgg

SEQ ID NO: 11 - DNA, 20 bp, synthetic construct
  source 1..20: mol_type = other DNA
aaacacgtggcaaacattcc

SEQ ID NO: 12 - DNA, 20 bp, synthetic construct
  source 1..20: mol_type = other DNA
aagaattactgacccctcgg

SEQ ID NO: 13 - DNA, 20 bp, synthetic construct
  source 1..20: mol_type = other DNA
aaagcactcttaggcctctg

SEQ ID NO: 14 - DNA, 20 bp, synthetic construct
  source 1..20: mol_type = other DNA
aaggactgcataccaggttg

SEQ ID NO: 15 - DNA, 20 bp, synthetic construct
  source 1..20: mol_type = other DNA
aaggcccagaaggatacaac

SEQ ID NO: 16 - DNA, 47 bp, synthetic construct
  source 1..47: mol_type = other DNA
gagatataaatatgnnbnnbnnbnnbnnbtagccgaccggcaccggc

SEQ ID NO: 17 - DNA, 53 bp, synthetic construct
  source 1..53: mol_type = other DNA
gagatataaatatgnnbnnbnnbnnbnnbnnbnnbtagccgaccggcaccggc

SEQ ID NO: 18 - DNA, 59 bp, synthetic construct
  source 1..59: mol_type = other DNA
gagatataaatatgnnbnnbnnbnnbnnbnnbnnbnnbnnbtagccgaccggcaccggc

SEQ ID NO: 19 - DNA, 65 bp, synthetic construct
  source 1..65: mol_type = other DNA
gagatataaatatgnnbnnbnnbnnbnnbnnbnnbnnbnnbnnbnnbtagccgaccggcaccggc

SEQ ID NO: 20 - DNA, 49 bp, synthetic construct
  source 1..49: mol_type = other DNA
gtaatacgactcactatagggttaactttaataaggagatataaatatg

SEQ ID NO: 21 - DNA, 95 bp, synthetic construct
  source 1..95: mol_type = other DNA
gtaatacgactcactatagggttaactttaataaggagatataaatatgnnbnnbnnbnnbnnbtagccgaccggcaccggcaccggcaaaaaaa

SEQ ID NO: 22 - DNA, 101 bp, synthetic construct
  source 1..101: mol_type = other DNA
gtaatacgactcactatagggttaactttaataaggagatataaatatgnnbnnbnnbnnbnnbnnbnnbtagccgaccggcaccggcaccggcaaaaaaa

SEQ ID NO: 23 - DNA, 107 bp, synthetic construct
  source 1..107: mol_type = other DNA
gtaatacgactcactatagggttaactttaataaggagatataaatatgnnbnnbnnbnnbnnbnnbnnbnnbnnbtagccgaccggcaccggcaccggcaaaaaaa

SEQ ID NO: 24 - DNA, 113 bp, synthetic construct
  source 1..113: mol_type = other DNA
gtaatacgactcactatagggttaactttaataaggagatataaatatgnnbnnbnnbnnbnnbnnbnnbnnbnnbnnbnnbtagccgaccggcaccggcaccggcaaaaaaa

SEQ ID NO: 25 - DNA, 60 bp, synthetic construct
  source 1..60: mol_type = other DNA
aaacacgtggcaaacattccaaaccggagccatacagtactttttttgccggtgccggtg

SEQ ID NO: 26 - DNA, 60 bp, synthetic construct
  source 1..60: mol_type = other DNA
aaacacgtggcaaacattccaacgatgatgctcactctcgtttttttgccggtgccggtg

SEQ ID NO: 27 - DNA, 60 bp, synthetic construct
  source 1..60: mol_type = other DNA
aaacacgtggcaaacattccaagacgatccgagccattactttttttgccggtgccggtg

SEQ ID NO: 28 - DNA, 20 bp, synthetic construct
  source 1..20: mol_type = other DNA
aaaccggagccatacagtac

SEQ ID NO: 29 - DNA, 20 bp, synthetic construct
  source 1..20: mol_type = other DNA
aacgatgatgctcactctcg

SEQ ID NO: 30 - DNA, 20 bp, synthetic construct
  source 1..20: mol_type = other DNA
aagacgatccgagccattac